European Patent Application EP 4 446 333 A1, published October 16, 2024. Title: 신규 아디포넥틴 유래 펩타이드 유도체 및 이의 용도. Applicant: 서울대학교병원. The sequence listing filed with the application follows.

SEQUENCE LISTING (16 sequences)

SEQ ID NO: 1 - protein, 4 aa, synthetic construct
DYYF

SEQ ID NO: 2 - protein, 5 aa, synthetic construct
GDFYF

SEQ ID NO: 3 - protein, 5 aa, synthetic construct
GDYFF

SEQ ID NO: 4 - protein, 5 aa, synthetic construct
GDYYF

SEQ ID NO: 5 - protein, 5 aa, synthetic construct
GDYYK

SEQ ID NO: 6 - protein, 5 aa, synthetic construct
GDYYY

SEQ ID NO: 7 - protein, 5 aa, synthetic construct
GEYYK

SEQ ID NO: 8 - protein, 5 aa, synthetic construct
GHYYF

SEQ ID NO: 9 - protein, 5 aa, synthetic construct
GIFYF

SEQ ID NO: 10 - protein, 5 aa, synthetic construct
GIWYF

SEQ ID NO: 11 - protein, 5 aa, synthetic construct
GIYYF

SEQ ID NO: 12 - protein, 5 aa, synthetic construct
GLFYF

SEQ ID NO: 13 - protein, 5 aa, synthetic construct
GLWYF

SEQ ID NO: 14 - protein, 5 aa, synthetic construct
GLYFF

SEQ ID NO: 15 - protein, 5 aa, synthetic construct
GLYYF

SEQ ID NO: 16 - protein, 5 aa, synthetic construct
GNYYF